European Patent Specification EP 3 558 369 B1, published March 26, 2025. Title: Antibodies that Specifically Bind to Human IL-15 and Uses Thereof. Applicant: Cephalon, Inc. The sequence listing filed with the application follows.

SEQUENCE LISTING (520 sequences)

SEQ ID NO: 1 - protein, 119 aa, Homo sapiens
  VARIANT (55)..(55): X is S, Y, W, or F
  VARIANT (57)..(57): X is N, Y, W, or F
  VARIANT (84)..(84): X is I or S
QVQLQESGPGLVKPSGTLSLTCAVSGGSISSSNWWSWVRQPPGKGLEWIGEIYHXGXTNYNPSLKSRVTISVDKSKNQFSLKLXSVTAADTAVYYCAREGIGWPSFDYWGQGTLVTVSS

SEQ ID NO: 2 - protein, 108 aa, Homo sapiens
  VARIANT (29)..(29): X is N or S
  VARIANT (92)..(92): X is S, L, or F
SSELTQDPAASVALGQTVRITCQGDTLRXYYASWYQQKPGQAPILVIYGKNNRPSGIPDRFSGSSSGNTASLTITGAQAEDEADYYCNSRDXSGKNLVFGGGTKLTVL

SEQ ID NO: 3 - protein, 214 aa, Homo sapiens
  VARIANT (29)..(29): X is N or S
  VARIANT (92)..(92): X is S, L, or F
SSELTQDPAASVALGQTVRITCQGDTLRXYYASWYQQKPGQAPILVIYGKNNRPSGIPDRFSGSSSGNTASLTITGAQAEDEADYYCNSRDXSGKNLVFGGGTKLTVLGQPKAAPSVTLFPPSSEELQANKATLVCLISDFYPGAVTVAWKADSSPVKAGVETTTPSKQSNNKYAASSYLSLTPEQWKSHRSYSCQVTHEGSTVEKTVAPTECS

SEQ ID NO: 4 - protein, 119 aa, Homo sapiens
QVQLQESGPGLVKPSGTLSLTCAVSGGSISSSNWWSWVRQPPGKGLEWIGEIYHYGYTNYNPSLKSRVTISVDKSKNQFSLKLSSVTAADTAVYYCAREGIGWPSFDYWGQGTLVTVSS

SEQ ID NO: 5 - protein, 108 aa, Homo sapiens
SSELTQDPAASVALGQTVRITCQGDTLRSYYASWYQQKPGQAPILVIYGKNNRPSGIPDRFSGSSSGNTASLTITGAQAEDEADYYCNSRDLSGKNLVFGGGTKLTVL

SEQ ID NO: 6 - protein, 214 aa, Homo sapiens
SSELTQDPAASVALGQTVRITCQGDTLRSYYASWYQQKPGQAPILVIYGKNNRPSGIPDRFSGSSSGNTASLTITGAQAEDEADYYCNSRDLSGKNLVFGGGTKLTVLGQPKAAPSVTLFPPSSEELQANKATLVCLISDFYPGAVTVAWKADSSPVKAGVETTTPSKQSNNKYAASSYLSLTPEQWKSHRSYSCQVTHEGSTVEKTVAPTECS

SEQ ID NO: 7 - protein, 119 aa, Homo sapiens
QVQLQESGPGLVKPSGTLSLTCAVSGGSISSSNWWSWVRQPPGKGLEWIGEIYHSGNTNYNPSLKSRVTISVDKSKNQFSLKLISVTAADTAVYYCAREGIGWPSFDYWGQGTLVTVSS

SEQ ID NO: 8 - protein, 108 aa, Homo sapiens
SSELTQDPAASVALGQTVRITCQGDTLRNYYASWYQQKPGQAPILVIYGKNNRPSGIPDRFSGSSSGNTASLTITGAQAEDEADYYCNSRDSSGKNLVFGGGTKLTVL

SEQ ID NO: 9 - protein, 214 aa, Homo sapiens
SSELTQDPAASVALGQTVRITCQGDTLRNYYASWYQQKPGQAPILVIYGKNNRPSGIPDRFSGSSSGNTASLTITGAQAEDEADYYCNSRDSSGKNLVFGGGTKLTVLGQPKAAPSVTLFPPSSEELQANKATLVCLISDFYPGAVTVAWKADSSPVKAGVETTTPSKQSNNKYAASSYLSLTPEQWKSHRSYSCQVTHEGSTVEKTVAPTECS

SEQ ID NO: 10 - protein, 30 aa, Homo sapiens
QVQLQESGPGLVKPSGTLSLTCAVSGGSIS

SEQ ID NO: 11 - protein, 14 aa, Homo sapiens
WVRQPPGKGLEWIG

SEQ ID NO: 12 - protein, 32 aa, Homo sapiens
  VARIANT (18)..(18): X is I or S
RVTISVDKSKNQFSLKLXSVTAADTAVYYCAR

SEQ ID NO: 13 - protein, 32 aa, Homo sapiens
RVTISVDKSKNQFSLKLSSVTAADTAVYYCAR

SEQ ID NO: 14 - protein, 32 aa, Homo sapiens
RVTISVDKSKNQFSLKLISVTAADTAVYYCAR

SEQ ID NO: 15 - protein, 11 aa, Homo sapiens
WGQGTLVTVSS

SEQ ID NO: 16 - protein, 6 aa, Homo sapiens
SSNWWS

SEQ ID NO: 17 - protein, 16 aa, Homo sapiens
  VARIANT (5)..(5): X is S, Y, W, or F
  VARIANT (7)..(7): X is N, Y, W, or F
EIYHXGXTNYNPSLKS

SEQ ID NO: 18 - protein, 16 aa, Homo sapiens
EIYHYGYTNYNPSLKS

SEQ ID NO: 19 - protein, 16 aa, Homo sapiens
EIYHSGNTNYNPSLKS

SEQ ID NO: 20 - protein, 10 aa, Homo sapiens
EGIGWPSFDY

SEQ ID NO: 21 - protein, 22 aa, Homo sapiens
SSELTQDPAASVALGQTVRITC

SEQ ID NO: 22 - protein, 15 aa, Homo sapiens
WYQQKPGQAPILVIY

SEQ ID NO: 23 - protein, 32 aa, Homo sapiens
GIPDRFSGSSSGNTASLTITGAQAEDEADYYC

SEQ ID NO: 24 - protein, 10 aa, Homo sapiens
FGGGTKLTVL

SEQ ID NO: 25 - protein, 11 aa, Homo sapiens
  VARIANT (7)..(7): X is N or S
QGDTLRXYYAS

SEQ ID NO: 26 - protein, 11 aa, Homo sapiens
QGDTLRSYYAS

SEQ ID NO: 27 - protein, 11 aa, Homo sapiens
QGDTLRNYYAS

SEQ ID NO: 28 - protein, 7 aa, Homo sapiens
GKNNRPS

SEQ ID NO: 29 - protein, 11 aa, Homo sapiens
  VARIANT (5)..(5): X is S, L, or F
NSRDXSGKNLV

SEQ ID NO: 30 - protein, 11 aa, Homo sapiens
NSRDLSGKNLV

SEQ ID NO: 31 - protein, 11 aa, Homo sapiens
NSRDSSGKNLV

SEQ ID NO: 32 - protein, 330 aa, Homo sapiens [sequence omitted]

SEQ ID NO: 33 - protein, 329 aa, Homo sapiens
ASTKGPSVFPLAPSSKSTSGGTAALGCLVKDYFPEPVTVSWNSGALTSGVHTFPAVLQSSGLYSLSSVVTVPSSSLGTQTYICNVNHKPSNTKVDKKVEPKSCDKTHTCPPCPAPELLGGPSVFLFPPKPKDTLMISRTPEVTCVVVDVSHEDPEVKFNWYVDGVEVHNAKTKPREEQYNSTYRVVSVLTVLHQDWLNGKEYKCKVSNKALPAPIEKTISKAKGQPREPQVYTLPPSRDELTKNQVSLTCLVKGFYPSDIAVEWESNGQPENNYKTTPPVLDSDGSFFLYSKLTVDKSRWQQGNVFSCSVMHEALHNHYTQKSLSLSPG

SEQ ID NO: 34 - protein, 330 aa, Homo sapiens
ASTKGPSVFPLAPSSKSTSGGTAALGCLVKDYFPEPVTVSWNSGALTSGVHTFPAVLQSSGLYSLSSVVTVPSSSLGTQTYICNVNHKPSNTKVDKKVEPKSCDKTHTCPPCPAPELLGGPSVFLFPPKPKDTLYITREPEVTCVVVDVSHEDPEVKFNWYVDGVEVHNAKTKPREEQYNSTYRVVSVLTVLHQDWLNGKEYKCKVSNKALPAPIEKTISKAKGQPREPQVYTLPPSRDELTKNQVSLTCLVKGFYPSDIAVEWESNGQPENNYKTTPPVLDSDGSFFLYSKLTVDKSRWQQGNVFSCSVMHEALHNHYTQKSLSLSPGK

SEQ ID NO: 35 - protein, 329 aa, Homo sapiens
ASTKGPSVFPLAPSSKSTSGGTAALGCLVKDYFPEPVTVSWNSGALTSGVHTFPAVLQSSGLYSLSSVVTVPSSSLGTQTYICNVNHKPSNTKVDKKVEPKSCDKTHTCPPCPAPELLGGPSVFLFPPKPKDTLYITREPEVTCVVVDVSHEDPEVKFNWYVDGVEVHNAKTKPREEQYNSTYRVVSVLTVLHQDWLNGKEYKCKVSNKALPAPIEKTISKAKGQPREPQVYTLPPSRDELTKNQVSLTCLVKGFYPSDIAVEWESNGQPENNYKTTPPVLDSDGSFFLYSKLTVDKSRWQQGNVFSCSVMHEALHNHYTQKSLSLSPG

SEQ ID NO: 36 - protein, 330 aa, Homo sapiens
ASTKGPSVFPLAPSSKSTSGGTAALGCLVKDYFPEPVTVSWNSGALTSGVHTFPAVLQSSGLYSLSSVVTVPSSSLGTQTYICNVNHKPSNTKVDKKVEPKSCDKTHTCPPCPAPELAGAPSVFLFPPKPKDTLMISRTPEVTCVVVDVSHEDPEVKFNWYVDGVEVHNAKTKPREEQYNSTYRVVSVLTVLHQDWLNGKEYKCKVSNKALPAPIEKTISKAKGQPREPQVYTLPPSRDELTKNQVSLTCLVKGFYPSDIAVEWESNGQPENNYKTTPPVLDSDGSFFLYSKLTVDKSRWQQGNVFSCSVMHEALHNHYTQKSLSLSPGK

SEQ ID NO: 37 - protein, 329 aa, Homo sapiens
ASTKGPSVFPLAPSSKSTSGGTAALGCLVKDYFPEPVTVSWNSGALTSGVHTFPAVLQSSGLYSLSSVVTVPSSSLGTQTYICNVNHKPSNTKVDKKVEPKSCDKTHTCPPCPAPELAGAPSVFLFPPKPKDTLMISRTPEVTCVVVDVSHEDPEVKFNWYVDGVEVHNAKTKPREEQYNSTYRVVSVLTVLHQDWLNGKEYKCKVSNKALPAPIEKTISKAKGQPREPQVYTLPPSRDELTKNQVSLTCLVKGFYPSDIAVEWESNGQPENNYKTTPPVLDSDGSFFLYSKLTVDKSRWQQGNVFSCSVMHEALHNHYTQKSLSLSPG

SEQ ID NO: 38 - protein, 330 aa, Homo sapiens
ASTKGPSVFPLAPSSKSTSGGTAALGCLVKDYFPEPVTVSWNSGALTSGVHTFPAVLQSSGLYSLSSVVTVPSSSLGTQTYICNVNHKPSNTKVDKKVEPKSCDKTHTCPPCPAPEAAGAPSVFLFPPKPKDTLMISRTPEVTCVVVDVSHEDPEVKFNWYVDGVEVHNAKTKPREEQYNSTYRVVSVLTVLHQDWLNGKEYKCKVSNKALPAPIEKTISKAKGQPREPQVYTLPPSREEMTKNQVSLTCLVKGFYPSDIAVEWESNGQPENNYKTTPPVLDSDGSFFLYSKLTVDKSRWQQGNVFSCSVMHEALHNHYTQKSLSLSPGK

SEQ ID NO: 39 - protein, 329 aa, Homo sapiens
ASTKGPSVFPLAPSSKSTSGGTAALGCLVKDYFPEPVTVSWNSGALTSGVHTFPAVLQSSGLYSLSSVVTVPSSSLGTQTYICNVNHKPSNTKVDKKVEPKSCDKTHTCPPCPAPEAAGAPSVFLFPPKPKDTLMISRTPEVTCVVVDVSHEDPEVKFNWYVDGVEVHNAKTKPREEQYNSTYRVVSVLTVLHQDWLNGKEYKCKVSNKALPAPIEKTISKAKGQPREPQVYTLPPSREEMTKNQVSLTCLVKGFYPSDIAVEWESNGQPENNYKTTPPVLDSDGSFFLYSKLTVDKSRWQQGNVFSCSVMHEALHNHYTQKSLSLSPG

SEQ ID NO: 40 - protein, 326 aa, Homo sapiens
ASTKGPSVFPLAPCSRSTSESTAALGCLVKDYFPEPVTVSWNSGALTSGVHTFPAVLQSSGLYSLSSVVTVPSSNFGTQTYTCNVDHKPSNTKVDKTVERKCCVECPPCPAPPVAGPSVFLFPPKPKDTLMISRTPEVTCVVVDVSHEDPEVQFNWYVDGVEVHNAKTKPREEQFNSTFRVVSVLTVVHQDWLNGKEYKCKVSNKGLPAPIEKTISKTKGQPREPQVYTLPPSREEMTKNQVSLTCLVKGFYPSDIAVEWESNGQPENNYKTTPPMLDSDGSFFLYSKLTVDKSRWQQGNVFSCSVMHEALHNHYTQKSLSLSPGK

SEQ ID NO: 41 - protein, 325 aa, Homo sapiens
ASTKGPSVFPLAPCSRSTSESTAALGCLVKDYFPEPVTVSWNSGALTSGVHTFPAVLQSSGLYSLSSVVTVPSSNFGTQTYTCNVDHKPSNTKVDKTVERKCCVECPPCPAPPVAGPSVFLFPPKPKDTLMISRTPEVTCVVVDVSHEDPEVQFNWYVDGVEVHNAKTKPREEQFNSTFRVVSVLTVVHQDWLNGKEYKCKVSNKGLPAPIEKTISKTKGQPREPQVYTLPPSREEMTKNQVSLTCLVKGFYPSDIAVEWESNGQPENNYKTTPPMLDSDGSFFLYSKLTVDKSRWQQGNVFSCSVMHEALHNHYTQKSLSLSPG

SEQ ID NO: 42 - protein, 326 aa, Homo sapiens
ASTKGPSVFPLAPCSRSTSESTAALGCLVKDYFPEPVTVSWNSGALTSGVHTFPAVLQSSGLYSLSSVVTVPSSNFGTQTYTCNVDHKPSNTKVDKTVERKCCVECPPCPAPPVAGPSVFLFPPKPKDTLMISRTPEVTCVVVDVSHEDPEVQFNWYVDGVEVHNAKTKPREEQFNSTFRVVSVLTVVHQDWLNGKEYKCKVSNKGLPSSIEKTISKTKGQPREPQVYTLPPSREEMTKNQVSLTCLVKGFYPSDIAVEWESNGQPENNYKTTPPMLDSDGSFFLYSKLTVDKSRWQQGNVFSCSVMHEALHNHYTQKSLSLSPGK

SEQ ID NO: 43 - protein, 325 aa, Homo sapiens
ASTKGPSVFPLAPCSRSTSESTAALGCLVKDYFPEPVTVSWNSGALTSGVHTFPAVLQSSGLYSLSSVVTVPSSNFGTQTYTCNVDHKPSNTKVDKTVERKCCVECPPCPAPPVAGPSVFLFPPKPKDTLMISRTPEVTCVVVDVSHEDPEVQFNWYVDGVEVHNAKTKPREEQFNSTFRVVSVLTVVHQDWLNGKEYKCKVSNKGLPSSIEKTISKTKGQPREPQVYTLPPSREEMTKNQVSLTCLVKGFYPSDIAVEWESNGQPENNYKTTPPMLDSDGSFFLYSKLTVDKSRWQQGNVFSCSVMHEALHNHYTQKSLSLSPG

SEQ ID NO: 44 - protein, 327 aa, Homo sapiens
ASTKGPSVFPLAPCSRSTSESTAALGCLVKDYFPEPVTVSWNSGALTSGVHTFPAVLQSSGLYSLSSVVTVPSSSLGTKTYTCNVDHKPSNTKVDKRVESKYGPPCPSCPAPEFLGGPSVFLFPPKPKDTLMISRTPEVTCVVVDVSQEDPEVQFNWYVDGVEVHNAKTKPREEQFNSTYRVVSVLTVLHQDWLNGKEYKCKVSNKGLPSSIEKTISKAKGQPREPQVYTLPPSQEEMTKNQVSLTCLVKGFYPSDIAVEWESNGQPENNYKTTPPVLDSDGSFFLYSRLTVDKSRWQEGNVFSCSVMHEALHNHYTQKSLSLSLGK

SEQ ID NO: 45 - protein, 326 aa, Homo sapiens
ASTKGPSVFPLAPCSRSTSESTAALGCLVKDYFPEPVTVSWNSGALTSGVHTFPAVLQSSGLYSLSSVVTVPSSSLGTKTYTCNVDHKPSNTKVDKRVESKYGPPCPSCPAPEFLGGPSVFLFPPKPKDTLMISRTPEVTCVVVDVSQEDPEVQFNWYVDGVEVHNAKTKPREEQFNSTYRVVSVLTVLHQDWLNGKEYKCKVSNKGLPSSIEKTISKAKGQPREPQVYTLPPSQEEMTKNQVSLTCLVKGFYPSDIAVEWESNGQPENNYKTTPPVLDSDGSFFLYSRLTVDKSRWQEGNVFSCSVMHEALHNHYTQKSLSLSLG

SEQ ID NO: 46 - protein, 327 aa, Homo sapiens
ASTKGPSVFPLAPCSRSTSESTAALGCLVKDYFPEPVTVSWNSGALTSGVHTFPAVLQSSGLYSLSSVVTVPSSSLGTKTYTCNVDHKPSNTKVDKRVESKYGPPCPPCPAPEFLGGPSVFLFPPKPKDTLMISRTPEVTCVVVDVSQEDPEVQFNWYVDGVEVHNAKTKPREEQFNSTYRVVSVLTVLHQDWLNGKEYKCKVSNKGLPSSIEKTISKAKGQPREPQVYTLPPSQEEMTKNQVSLTCLVKGFYPSDIAVEWESNGQPENNYKTTPPVLDSDGSFFLYSRLTVDKSRWQEGNVFSCSVMHEALHNHYTQKSLSLSLGK

SEQ ID NO: 47 - protein, 326 aa, Homo sapiens
ASTKGPSVFPLAPCSRSTSESTAALGCLVKDYFPEPVTVSWNSGALTSGVHTFPAVLQSSGLYSLSSVVTVPSSSLGTKTYTCNVDHKPSNTKVDKRVESKYGPPCPPCPAPEFLGGPSVFLFPPKPKDTLMISRTPEVTCVVVDVSQEDPEVQFNWYVDGVEVHNAKTKPREEQFNSTYRVVSVLTVLHQDWLNGKEYKCKVSNKGLPSSIEKTISKAKGQPREPQVYTLPPSQEEMTKNQVSLTCLVKGFYPSDIAVEWESNGQPENNYKTTPPVLDSDGSFFLYSRLTVDKSRWQEGNVFSCSVMHEALHNHYTQKSLSLSLG

SEQ ID NO: 48 - protein, 327 aa, Homo sapiens
ASTKGPSVFPLAPCSRSTSESTAALGCLVKDYFPEPVTVSWNSGALTSGVHTFPAVLQSSGLYSLSSVVTVPSSSLGTKTYTCNVDHKPSNTKVDKRVESKYGPPCPPCPAPEFLGGPSVFLFPPKPKDTLYITREPEVTCVVVDVSQEDPEVQFNWYVDGVEVHNAKTKPREEQFNSTYRVVSVLTVLHQDWLNGKEYKCKVSNKGLPSSIEKTISKAKGQPREPQVYTLPPSQEEMTKNQVSLTCLVKGFYPSDIAVEWESNGQPENNYKTTPPVLDSDGSFFLYSRLTVDKSRWQEGNVFSCSVMHEALHNHYTQKSLSLSLGK

SEQ ID NO: 49 - protein, 326 aa, Homo sapiens
ASTKGPSVFPLAPCSRSTSESTAALGCLVKDYFPEPVTVSWNSGALTSGVHTFPAVLQSSGLYSLSSVVTVPSSSLGTKTYTCNVDHKPSNTKVDKRVESKYGPPCPPCPAPEFLGGPSVFLFPPKPKDTLYITREPEVTCVVVDVSQEDPEVQFNWYVDGVEVHNAKTKPREEQFNSTYRVVSVLTVLHQDWLNGKEYKCKVSNKGLPSSIEKTISKAKGQPREPQVYTLPPSQEEMTKNQVSLTCLVKGFYPSDIAVEWESNGQPENNYKTTPPVLDSDGSFFLYSRLTVDKSRWQEGNVFSCSVMHEALHNHYTQKSLSLSLG

SEQ ID NO: 50 - protein, 327 aa, Homo sapiens
ASTKGPSVFPLAPCSRSTSESTAALGCLVKDYFPEPVTVSWNSGALTSGVHTFPAVLQSSGLYSLSSVVTVPSSSLGTKTYTCNVDHKPSNTKVDKRVESKYGPPCPSCPAPEFLGGPSVFLFPPKPKDTLYITREPEVTCVVVDVSQEDPEVQFNWYVDGVEVHNAKTKPREEQFNSTYRVVSVLTVLHQDWLNGKEYKCKVSNKGLPSSIEKTISKAKGQPREPQVYTLPPSQEEMTKNQVSLTCLVKGFYPSDIAVEWESNGQPENNYKTTPPVLDSDGSFFLYSRLTVDKSRWQEGNVFSCSVMHEALHNHYTQKSLSLSLGK

SEQ ID NO: 51 - protein, 326 aa, Homo sapiens
ASTKGPSVFPLAPCSRSTSESTAALGCLVKDYFPEPVTVSWNSGALTSGVHTFPAVLQSSGLYSLSSVVTVPSSSLGTKTYTCNVDHKPSNTKVDKRVESKYGPPCPSCPAPEFLGGPSVFLFPPKPKDTLYITREPEVTCVVVDVSQEDPEVQFNWYVDGVEVHNAKTKPREEQFNSTYRVVSVLTVLHQDWLNGKEYKCKVSNKGLPSSIEKTISKAKGQPREPQVYTLPPSQEEMTKNQVSLTCLVKGFYPSDIAVEWESNGQPENNYKTTPPVLDSDGSFFLYSRLTVDKSRWQEGNVFSCSVMHEALHNHYTQKSLSLSLG

SEQ ID NO: 52 - protein, 6 aa, Homo sapiens
ASNWWS

SEQ ID NO: 53 - protein, 6 aa, Homo sapiens
SANWWS

SEQ ID NO: 54 - protein, 6 aa, Homo sapiens
SSAWWS

SEQ ID NO: 55 - protein, 6 aa, Homo sapiens
SSNAWS

SEQ ID NO: 56 - protein, 6 aa, Homo sapiens
SSNWAS

SEQ ID NO: 57 - protein, 6 aa, Homo sapiens
SSNWWA

SEQ ID NO: 58 - protein, 11 aa, Homo sapiens
GASISSSNWWS

SEQ ID NO: 59 - protein, 11 aa, Homo sapiens
GGAISSSNWWS

SEQ ID NO: 60 - protein, 11 aa, Homo sapiens
GGSASSSNWWS

SEQ ID NO: 61 - protein, 11 aa, Homo sapiens
GGSIASSNWWS

SEQ ID NO: 62 - protein, 11 aa, Homo sapiens
GGSISASNWWS

SEQ ID NO: 63 - protein, 11 aa, Homo sapiens
GGSISSANWWS

SEQ ID NO: 64 - protein, 11 aa, Homo sapiens
GGSISSSAWWS

SEQ ID NO: 65 - protein, 11 aa, Homo sapiens
GGSISSSNWWA

SEQ ID NO: 66 - protein, 11 aa, Homo sapiens
DGSISSSNWWS

SEQ ID NO: 67 - protein, 11 aa, Homo sapiens
GDSISSSNWWS

SEQ ID NO: 68 - protein, 11 aa, Homo sapiens
GGDISSSNWWS

SEQ ID NO: 69 - protein, 11 aa, Homo sapiens
GGSDSSSNWWS

SEQ ID NO: 70 - protein, 11 aa, Homo sapiens
GGSIDSSNWWS

SEQ ID NO: 71 - protein, 11 aa, Homo sapiens
GGSISDSNWWS

SEQ ID NO: 72 - protein, 11 aa, Homo sapiens
GGSISSDNWWS

SEQ ID NO: 73 - protein, 11 aa, Homo sapiens
GGSISSSDWWS

SEQ ID NO: 74 - protein, 11 aa, Homo sapiens
GGSISSSNDWS

SEQ ID NO: 75 - protein, 11 aa, Homo sapiens
GGSISSSNWWD

SEQ ID NO: 76 - protein, 11 aa, Homo sapiens
HGSISSSNWWS

SEQ ID NO: 77 - protein, 11 aa, Homo sapiens
GHSISSSNWWS

SEQ ID NO: 78 - protein, 11 aa, Homo sapiens
GGHISSSNWWS

SEQ ID NO: 79 - protein, 11 aa, Homo sapiens
GGSHSSSNWWS

SEQ ID NO: 80 - protein, 11 aa, Homo sapiens
GGSIHSSNWWS

SEQ ID NO: 81 - protein, 11 aa, Homo sapiens
GGSISHSNWWS

SEQ ID NO: 82 - protein, 11 aa, Homo sapiens
GGSISSHNWWS

SEQ ID NO: 83 - protein, 11 aa, Homo sapiens
GGSISSSHWWS

SEQ ID NO: 84 - protein, 11 aa, Homo sapiens
GGSISSSNHWS

SEQ ID NO: 85 - protein, 11 aa, Homo sapiens
GGSISSSNWHS

SEQ ID NO: 86 - protein, 11 aa, Homo sapiens
KGSISSSNWWS

SEQ ID NO: 87 - protein, 11 aa, Homo sapiens
GKSISSSNWWS

SEQ ID NO: 88 - protein, 11 aa, Homo sapiens
GGKISSSNWWS

SEQ ID NO: 89 - protein, 11 aa, Homo sapiens
GGSKSSSNWWS

SEQ ID NO: 90 - protein, 11 aa, Homo sapiens
GGSIKSSNWWS

SEQ ID NO: 91 - protein, 11 aa, Homo sapiens
GGSISKSNWWS

SEQ ID NO: 92 - protein, 11 aa, Homo sapiens
GGSISSKNWWS

SEQ ID NO: 93 - protein, 11 aa, Homo sapiens
LGSISSSNWWS

SEQ ID NO: 94 - protein, 11 aa, Homo sapiens
GLSISSSNWWS

SEQ ID NO: 95 - protein, 11 aa, Homo sapiens
GGLISSSNWWS

SEQ ID NO: 96 - protein, 11 aa, Homo sapiens
GGSLSSSNWWS

SEQ ID NO: 97 - protein, 11 aa, Homo sapiens
GGSILSSNWWS

SEQ ID NO: 98 - protein, 11 aa, Homo sapiens
GGSISLSNWWS

SEQ ID NO: 99 - protein, 11 aa, Homo sapiens
GGSISSLNWWS

SEQ ID NO: 100 - protein, 11 aa, Homo sapiens
GGSISSSLWWS

SEQ ID NO: 101 - protein, 11 aa, Homo sapiens
GGSISSSNLWS

SEQ ID NO: 102 - protein, 11 aa, Homo sapiens
GGSISSSNWLS

SEQ ID NO: 103 - protein, 11 aa, Homo sapiens
GGSISSSNWWL

SEQ ID NO: 104 - protein, 11 aa, Homo sapiens
QGSISSSNWWS

SEQ ID NO: 105 - protein, 11 aa, Homo sapiens
GQSISSSNWWS

SEQ ID NO: 106 - protein, 11 aa, Homo sapiens
GGQISSSNWWS

SEQ ID NO: 107 - protein, 11 aa, Homo sapiens
GGSQSSSNWWS

SEQ ID NO: 108 - protein, 11 aa, Homo sapiens
GGSIQSSNWWS

SEQ ID NO: 109 - protein, 11 aa, Homo sapiens
GGSISQSNWWS

SEQ ID NO: 110 - protein, 11 aa, Homo sapiens
GGSISSQNWWS

SEQ ID NO: 111 - protein, 11 aa, Homo sapiens
GGSISSSQWWS

SEQ ID NO: 112 - protein, 11 aa, Homo sapiens
GGSISSSNQWS

SEQ ID NO: 113 - protein, 11 aa, Homo sapiens
SGSISSSNWWS

SEQ ID NO: 114 - protein, 11 aa, Homo sapiens
GSSISSSNWWS

SEQ ID NO: 115 - protein, 11 aa, Homo sapiens
GGSSSSSNWWS

SEQ ID NO: 116 - protein, 11 aa, Homo sapiens
GGSISSSSWWS

SEQ ID NO: 117 - protein, 11 aa, Homo sapiens
GGSISSSNSWS

SEQ ID NO: 118 - protein, 11 aa, Homo sapiens
WGSISSSNWWS

SEQ ID NO: 119 - protein, 11 aa, Homo sapiens
GWSISSSNWWS

SEQ ID NO: 120 - protein, 11 aa, Homo sapiens
GGWISSSNWWS

SEQ ID NO: 121 - protein, 11 aa, Homo sapiens
GGSWSSSNWWS

SEQ ID NO: 122 - protein, 11 aa, Homo sapiens
GGSIWSSNWWS

SEQ ID NO: 123 - protein, 11 aa, Homo sapiens
GGSISWSNWWS

SEQ ID NO: 124 - protein, 11 aa, Homo sapiens
GGSISSWNWWS

SEQ ID NO: 125 - protein, 11 aa, Homo sapiens
GGSISSSWWWS

SEQ ID NO: 126 - protein, 11 aa, Homo sapiens
YGSISSSNWWS

SEQ ID NO: 127 - protein, 11 aa, Homo sapiens
GYSISSSNWWS

SEQ ID NO: 128 - protein, 11 aa, Homo sapiens
GGYISSSNWWS

SEQ ID NO: 129 - protein, 11 aa, Homo sapiens
GGSYSSSNWWS

SEQ ID NO: 130 - protein, 11 aa, Homo sapiens
GGSIYSSNWWS

SEQ ID NO: 131 - protein, 11 aa, Homo sapiens
GGSISYSNWWS

SEQ ID NO: 132 - protein, 11 aa, Homo sapiens
GGSISSYNWWS

SEQ ID NO: 133 - protein, 11 aa, Homo sapiens
GGSISSSYWWS

SEQ ID NO: 134 - protein, 11 aa, Homo sapiens
GGSISSSNYWS

SEQ ID NO: 135 - protein, 11 aa, Homo sapiens
GGSISSSNWYS

SEQ ID NO: 136 - protein, 11 aa, Homo sapiens
AIYHSGNTNYN

SEQ ID NO: 137 - protein, 11 aa, Homo sapiens
EAYHSGNTNYN

SEQ ID NO: 138 - protein, 11 aa, Homo sapiens
EIAHSGNTNYN

SEQ ID NO: 139 - protein, 11 aa, Homo sapiens
EIYASGNTNYN

SEQ ID NO: 140 - protein, 11 aa, Homo sapiens
EIYHAGNTNYN

SEQ ID NO: 141 - protein, 11 aa, Homo sapiens
EIYHSANTNYN

SEQ ID NO: 142 - protein, 11 aa, Homo sapiens
EIYHSGATNYN

SEQ ID NO: 143 - protein, 11 aa, Homo sapiens
EIYHSGNANYN

SEQ ID NO: 144 - protein, 11 aa, Homo sapiens
EIYHSGNTAYN

SEQ ID NO: 145 - protein, 11 aa, Homo sapiens
EIYHSGNTNAN

SEQ ID NO: 146 - protein, 11 aa, Homo sapiens
EIYHSGNTNYA

SEQ ID NO: 147 - protein, 11 aa, Homo sapiens
DIYHSGNTNYN

SEQ ID NO: 148 - protein, 11 aa, Homo sapiens
EIDHSGNTNYN

SEQ ID NO: 149 - protein, 11 aa, Homo sapiens
EIYDSGNTNYN

SEQ ID NO: 150 - protein, 11 aa, Homo sapiens
EIYHDGNTNYN

SEQ ID NO: 151 - protein, 11 aa, Homo sapiens
EIYHSGDTNYN

SEQ ID NO: 152 - protein, 11 aa, Homo sapiens
EIYHSGNDNYN

SEQ ID NO: 153 - protein, 11 aa, Homo sapiens
EIYHSGNTDYN

SEQ ID NO: 154 - protein, 11 aa, Homo sapiens
EIYHSGNTNDN

SEQ ID NO: 155 - protein, 11 aa, Homo sapiens
EIYHSGNTNYD

SEQ ID NO: 156 - protein, 11 aa, Homo sapiens
HIYHSGNTNYN

SEQ ID NO: 157 - protein, 11 aa, Homo sapiens
EHYHSGNTNYN

SEQ ID NO: 158 - protein, 11 aa, Homo sapiens
EIHHSGNTNYN

SEQ ID NO: 159 - protein, 11 aa, Homo sapiens
EIYHHGNTNYN

SEQ ID NO: 160 - protein, 11 aa, Homo sapiens
EIYHSHNTNYN

SEQ ID NO: 161 - protein, 11 aa, Homo sapiens
EIYHSGHTNYN

SEQ ID NO: 162 - protein, 11 aa, Homo sapiens
EIYHSGNHNYN

SEQ ID NO: 163 - protein, 11 aa, Homo sapiens
EIYHSGNTHYN

SEQ ID NO: 164 - protein, 11 aa, Homo sapiens
EIYHSGNTNHN

SEQ ID NO: 165 - protein, 11 aa, Homo sapiens
EIYHSGNTNYH

SEQ ID NO: 166 - protein, 11 aa, Homo sapiens
EKYHSGNTNYN

SEQ ID NO: 167 - protein, 11 aa, Homo sapiens
EIKHSGNTNYN

SEQ ID NO: 168 - protein, 11 aa, Homo sapiens
EIYKSGNTNYN

SEQ ID NO: 169 - protein, 11 aa, Homo sapiens
EIYHKGNTNYN

SEQ ID NO: 170 - protein, 11 aa, Homo sapiens
EIYHSKNTNYN

SEQ ID NO: 171 - protein, 11 aa, Homo sapiens
EIYHSGKTNYN

SEQ ID NO: 172 - protein, 11 aa, Homo sapiens
EIYHSGNKNYN

SEQ ID NO: 173 - protein, 11 aa, Homo sapiens
EIYHSGNTKYN

SEQ ID NO: 174 - protein, 11 aa, Homo sapiens
EIYHSGNTNKN

SEQ ID NO: 175 - protein, 11 aa, Homo sapiens
EIYHSGNTNYK

SEQ ID NO: 176 - protein, 11 aa, Homo sapiens
LIYHSGNTNYN

SEQ ID NO: 177 - protein, 11 aa, Homo sapiens
ELYHSGNTNYN

SEQ ID NO: 178 - protein, 11 aa, Homo sapiens
EILHSGNTNYN

SEQ ID NO: 179 - protein, 11 aa, Homo sapiens
EIYLSGNTNYN

SEQ ID NO: 180 - protein, 11 aa, Homo sapiens
EIYHLGNTNYN

SEQ ID NO: 181 - protein, 11 aa, Homo sapiens
EIYHSLNTNYN

SEQ ID NO: 182 - protein, 11 aa, Homo sapiens
EIYHSGLTNYN

SEQ ID NO: 183 - protein, 11 aa, Homo sapiens
EIYHSGNLNYN

SEQ ID NO: 184 - protein, 11 aa, Homo sapiens
EIYHSGNTLYN

SEQ ID NO: 185 - protein, 11 aa, Homo sapiens
EIYHSGNTNLN

SEQ ID NO: 186 - protein, 11 aa, Homo sapiens
EIYHSGNTNYL

SEQ ID NO: 187 - protein, 11 aa, Homo sapiens
QIYHSGNTNYN

SEQ ID NO: 188 - protein, 11 aa, Homo sapiens
EQYHSGNTNYN

SEQ ID NO: 189 - protein, 11 aa, Homo sapiens
EIQHSGNTNYN

SEQ ID NO: 190 - protein, 11 aa, Homo sapiens
EIYQSGNTNYN

SEQ ID NO: 191 - protein, 11 aa, Homo sapiens
EIYHQGNTNYN

SEQ ID NO: 192 - protein, 11 aa, Homo sapiens
EIYHSQNTNYN

SEQ ID NO: 193 - protein, 11 aa, Homo sapiens
EIYHSGQTNYN

SEQ ID NO: 194 - protein, 11 aa, Homo sapiens
EIYHSGNQNYN

SEQ ID NO: 195 - protein, 11 aa, Homo sapiens
EIYHSGNTQYN

SEQ ID NO: 196 - protein, 11 aa, Homo sapiens
EIYHSGNTNQN

SEQ ID NO: 197 - protein, 11 aa, Homo sapiens
EIYHSGNTNYQ

SEQ ID NO: 198 - protein, 11 aa, Homo sapiens
SIYHSGNTNYN

SEQ ID NO: 199 - protein, 11 aa, Homo sapiens
ESYHSGNTNYN

SEQ ID NO: 200 - protein, 11 aa, Homo sapiens
EISHSGNTNYN

SEQ ID NO: 201 - protein, 11 aa, Homo sapiens
EIYSSGNTNYN

SEQ ID NO: 202 - protein, 11 aa, Homo sapiens
EIYHSSNTNYN

SEQ ID NO: 203 - protein, 11 aa, Homo sapiens
EIYHSGSTNYN

SEQ ID NO: 204 - protein, 11 aa, Homo sapiens
EIYHSGNSNYN

SEQ ID NO: 205 - protein, 11 aa, Homo sapiens
EIYHSGNTSYN

SEQ ID NO: 206 - protein, 11 aa, Homo sapiens
EIYHSGNTNSN

SEQ ID NO: 207 - protein, 11 aa, Homo sapiens
EIYHSGNTNYS

SEQ ID NO: 208 - protein, 11 aa, Homo sapiens
WIYHSGNTNYN

SEQ ID NO: 209 - protein, 11 aa, Homo sapiens
EIWHSGNTNYN

SEQ ID NO: 210 - protein, 11 aa, Homo sapiens
EIYWSGNTNYN

SEQ ID NO: 211 - protein, 11 aa, Homo sapiens
EIYHWGNTNYN

SEQ ID NO: 212 - protein, 11 aa, Homo sapiens
EIYHSWNTNYN

SEQ ID NO: 213 - protein, 11 aa, Homo sapiens
EIYHSGWTNYN

SEQ ID NO: 214 - protein, 11 aa, Homo sapiens
EIYHSGNWNYN

SEQ ID NO: 215 - protein, 11 aa, Homo sapiens
EIYHSGNTWYN

SEQ ID NO: 216 - protein, 11 aa, Homo sapiens
EIYHSGNTNWN

SEQ ID NO: 217 - protein, 11 aa, Homo sapiens
EIYHSGNTNYW

SEQ ID NO: 218 - protein, 11 aa, Homo sapiens
YIYHSGNTNYN

SEQ ID NO: 219 - protein, 11 aa, Homo sapiens
EYYHSGNTNYN

SEQ ID NO: 220 - protein, 11 aa, Homo sapiens
EIYYSGNTNYN

SEQ ID NO: 221 - protein, 11 aa, Homo sapiens
EIYHYGNTNYN

SEQ ID NO: 222 - protein, 11 aa, Homo sapiens
EIYHSYNTNYN

SEQ ID NO: 223 - protein, 11 aa, Homo sapiens
EIYHSGYTNYN

SEQ ID NO: 224 - protein, 11 aa, Homo sapiens
EIYHSGNYNYN

SEQ ID NO: 225 - protein, 11 aa, Homo sapiens
EIYHSGNTYYN

SEQ ID NO: 226 - protein, 11 aa, Homo sapiens
EIYHSGNTNYY

SEQ ID NO: 227 - protein, 10 aa, Homo sapiens
AGIGWPSFDY

SEQ ID NO: 228 - protein, 10 aa, Homo sapiens
EAIGWPSFDY

SEQ ID NO: 229 - protein, 10 aa, Homo sapiens
EGAGWPSFDY

SEQ ID NO: 230 - protein, 10 aa, Homo sapiens
EGIAWPSFDY

SEQ ID NO: 231 - protein, 10 aa, Homo sapiens
EGIGWPAFDY

SEQ ID NO: 232 - protein, 10 aa, Homo sapiens
EGIGWPSFDA

SEQ ID NO: 233 - protein, 10 aa, Homo sapiens
DGIGWPSFDY

SEQ ID NO: 234 - protein, 10 aa, Homo sapiens
EDIGWPSFDY

SEQ ID NO: 235 - protein, 10 aa, Homo sapiens
EGDGWPSFDY

SEQ ID NO: 236 - protein, 10 aa, Homo sapiens
EGIGWPSFDD

SEQ ID NO: 237 - protein, 10 aa, Homo sapiens
HGIGWPSFDY

SEQ ID NO: 238 - protein, 10 aa, Homo sapiens
EHIGWPSFDY

SEQ ID NO: 239 - protein, 10 aa, Homo sapiens
EGHGWPSFDY

SEQ ID NO: 240 - protein, 10 aa, Homo sapiens
EGIGWPHFDY

SEQ ID NO: 241 - protein, 10 aa, Homo sapiens
EGIGWPSHDY

SEQ ID NO: 242 - protein, 10 aa, Homo sapiens
EGIGWPSFDH

SEQ ID NO: 243 - protein, 10 aa, Homo sapiens
EKIGWPSFDY

SEQ ID NO: 244 - protein, 10 aa, Homo sapiens
EGKGWPSFDY

SEQ ID NO: 245 - protein, 10 aa, Homo sapiens
EGIGWPSFKY

SEQ ID NO: 246 - protein, 10 aa, Homo sapiens
EGIGWPSFDK

SEQ ID NO: 247 - protein, 10 aa, Homo sapiens
LGIGWPSFDY

SEQ ID NO: 248 - protein, 10 aa, Homo sapiens
EGLGWPSFDY

SEQ ID NO: 249 - protein, 10 aa, Homo sapiens
EGIGWPLFDY

SEQ ID NO: 250 - protein, 10 aa, Homo sapiens
EGIGWPSLDY

SEQ ID NO: 251 - protein, 10 aa, Homo sapiens
EGIGWPSFDL

SEQ ID NO: 252 - protein, 10 aa, Homo sapiens
QGIGWPSFDY

SEQ ID NO: 253 - protein, 10 aa, Homo sapiens
EQIGWPSFDY

SEQ ID NO: 254 - protein, 10 aa, Homo sapiens
EGQGWPSFDY

SEQ ID NO: 255 - protein, 10 aa, Homo sapiens
EGIGWPQFDY

SEQ ID NO: 256 - protein, 10 aa, Homo sapiens
EGIGWPSFQY

SEQ ID NO: 257 - protein, 10 aa, Homo sapiens
EGIGWPSFDQ

SEQ ID NO: 258 - protein, 10 aa, Homo sapiens
SGIGWPSFDY

SEQ ID NO: 259 - protein, 10 aa, Homo sapiens
ESIGWPSFDY

SEQ ID NO: 260 - protein, 10 aa, Homo sapiens
EGSGWPSFDY

SEQ ID NO: 261 - protein, 10 aa, Homo sapiens
EGIGWPSFDS

SEQ ID NO: 262 - protein, 10 aa, Homo sapiens
EWIGWPSFDY

SEQ ID NO: 263 - protein, 10 aa, Homo sapiens
EGWGWPSFDY

SEQ ID NO: 264 - protein, 10 aa, Homo sapiens
EGIGWPWFDY

SEQ ID NO: 265 - protein, 10 aa, Homo sapiens
EGIGWPSWDY

SEQ ID NO: 266 - protein, 10 aa, Homo sapiens
EGIGWPSFDW

SEQ ID NO: 267 - protein, 10 aa, Homo sapiens
EYIGWPSFDY

SEQ ID NO: 268 - protein, 10 aa, Homo sapiens
EGYGWPSFDY

SEQ ID NO: 269 - protein, 10 aa, Homo sapiens
EGIGYPSFDY

SEQ ID NO: 270 - protein, 10 aa, Homo sapiens
EGIGWPYFDY

SEQ ID NO: 271 - protein, 10 aa, Homo sapiens
EGIGWPSYDY

SEQ ID NO: 272 - protein, 10 aa, Homo sapiens
EGIGWPSFYY

SEQ ID NO: 273 - protein, 11 aa, Homo sapiens
AGDTLRNYYAS

SEQ ID NO: 274 - protein, 11 aa, Homo sapiens
QADTLRNYYAS

SEQ ID NO: 275 - protein, 11 aa, Homo sapiens
QGATLRNYYAS

SEQ ID NO: 276 - protein, 11 aa, Homo sapiens
QGDALRNYYAS

SEQ ID NO: 277 - protein, 11 aa, Homo sapiens
QGDTARNYYAS

SEQ ID NO: 278 - protein, 11 aa, Homo sapiens
QGDTLANYYAS

SEQ ID NO: 279 - protein, 11 aa, Homo sapiens
QGDTLRAYYAS

SEQ ID NO: 280 - protein, 11 aa, Homo sapiens
QGDTLRNYAAS

SEQ ID NO: 281 - protein, 11 aa, Homo sapiens
QGDTLRNYYAA

SEQ ID NO: 282 - protein, 11 aa, Homo sapiens
DGDTLRNYYAS

SEQ ID NO: 283 - protein, 11 aa, Homo sapiens
QDDTLRNYYAS

SEQ ID NO: 284 - protein, 11 aa, Homo sapiens
QGDDLRNYYAS

SEQ ID NO: 285 - protein, 11 aa, Homo sapiens
QGDTLDNYYAS

SEQ ID NO: 286 - protein, 11 aa, Homo sapiens
QGDTLRDYYAS

SEQ ID NO: 287 - protein, 11 aa, Homo sapiens
HGDTLRNYYAS

SEQ ID NO: 288 - protein, 11 aa, Homo sapiens
QHDTLRNYYAS

SEQ ID NO: 289 - protein, 11 aa, Homo sapiens
QGHTLRNYYAS

SEQ ID NO: 290 - protein, 11 aa, Homo sapiens
QGDHLRNYYAS

SEQ ID NO: 291 - protein, 11 aa, Homo sapiens
QGDTHRNYYAS

SEQ ID NO: 292 - protein, 11 aa, Homo sapiens
QGDTLHNYYAS

SEQ ID NO: 293 - protein, 11 aa, Homo sapiens
QGDTLRHYYAS

SEQ ID NO: 294 - protein, 11 aa, Homo sapiens
QGDTLRNYHAS

SEQ ID NO: 295 - protein, 11 aa, Homo sapiens
KGDTLRNYYAS

SEQ ID NO: 296 - protein, 11 aa, Homo sapiens
QKDTLRNYYAS

SEQ ID NO: 297 - protein, 11 aa, Homo sapiens
QGKTLRNYYAS

SEQ ID NO: 298 - protein, 11 aa, Homo sapiens
QGDTLKNYYAS

SEQ ID NO: 299 - protein, 11 aa, Homo sapiens
QGDTLRKYYAS

SEQ ID NO: 300 - protein, 11 aa, Homo sapiens
LGDTLRNYYAS

SEQ ID NO: 301 - protein, 11 aa, Homo sapiens
QGLTLRNYYAS

SEQ ID NO: 302 - protein, 11 aa, Homo sapiens
QGDLLRNYYAS

SEQ ID NO: 303 - protein, 11 aa, Homo sapiens
QGDTLLNYYAS

SEQ ID NO: 304 - protein, 11 aa, Homo sapiens
QGDTLRLYYAS

SEQ ID NO: 305 - protein, 11 aa, Homo sapiens
QGDTLRNYLAS

SEQ ID NO: 306 - protein, 11 aa, Homo sapiens
QQDTLRNYYAS

SEQ ID NO: 307 - protein, 11 aa, Homo sapiens
QGQTLRNYYAS

SEQ ID NO: 308 - protein, 11 aa, Homo sapiens
QGDQLRNYYAS

SEQ ID NO: 309 - protein, 11 aa, Homo sapiens
QGDTLQNYYAS

SEQ ID NO: 310 - protein, 11 aa, Homo sapiens
QGDTLRQYYAS

SEQ ID NO: 311 - protein, 11 aa, Homo sapiens
QGDTLRNYQAS

SEQ ID NO: 312 - protein, 11 aa, Homo sapiens
SGDTLRNYYAS

SEQ ID NO: 313 - protein, 11 aa, Homo sapiens
QSDTLRNYYAS

SEQ ID NO: 314 - protein, 11 aa, Homo sapiens
QGSTLRNYYAS

SEQ ID NO: 315 - protein, 11 aa, Homo sapiens
QGDSLRNYYAS

SEQ ID NO: 316 - protein, 11 aa, Homo sapiens
QGDTLSNYYAS

SEQ ID NO: 317 - protein, 11 aa, Homo sapiens
QGDTLRSYYAS

SEQ ID NO: 318 - protein, 11 aa, Homo sapiens
WGDTLRNYYAS

SEQ ID NO: 319 - protein, 11 aa, Homo sapiens
QGWTLRNYYAS

SEQ ID NO: 320 - protein, 11 aa, Homo sapiens
QGDWLRNYYAS

SEQ ID NO: 321 - protein, 11 aa, Homo sapiens
QGDTLWNYYAS

SEQ ID NO: 322 - protein, 11 aa, Homo sapiens
QGDTLRWYYAS

SEQ ID NO: 323 - protein, 11 aa, Homo sapiens
QGDTLRNWYAS

SEQ ID NO: 324 - protein, 11 aa, Homo sapiens
QGDTLRNYWAS

SEQ ID NO: 325 - protein, 11 aa, Homo sapiens
YGDTLRNYYAS

SEQ ID NO: 326 - protein, 11 aa, Homo sapiens
QGYTLRNYYAS

SEQ ID NO: 327 - protein, 11 aa, Homo sapiens
QGDYLRNYYAS

SEQ ID NO: 328 - protein, 11 aa, Homo sapiens
QGDTLYNYYAS

SEQ ID NO: 329 - protein, 11 aa, Homo sapiens
QGDTLRYYYAS

SEQ ID NO: 330 - protein, 7 aa, Homo sapiens
AKNNRPS

SEQ ID NO: 331 - protein, 7 aa, Homo sapiens
GANNRPS

SEQ ID NO: 332 - protein, 7 aa, Homo sapiens
GKANRPS

SEQ ID NO: 333 - protein, 7 aa, Homo sapiens
GKNARPS

SEQ ID NO: 334 - protein, 7 aa, Homo sapiens
GKNNAPS

SEQ ID NO: 335 - protein, 7 aa, Homo sapiens
GKNNRAS

SEQ ID NO: 336 - protein, 7 aa, Homo sapiens
GKNNRPA

SEQ ID NO: 337 - protein, 7 aa, Homo sapiens
DKNNRPS

SEQ ID NO: 338 - protein, 7 aa, Homo sapiens
GDNNRPS

SEQ ID NO: 339 - protein, 7 aa, Homo sapiens
GKDNRPS

SEQ ID NO: 340 - protein, 7 aa, Homo sapiens
GKNDRPS

SEQ ID NO: 341 - protein, 7 aa, Homo sapiens
GKNNDPS

SEQ ID NO: 342 - protein, 7 aa, Homo sapiens
GKNNRDS

SEQ ID NO: 343 - protein, 7 aa, Homo sapiens
GKNNRPD

SEQ ID NO: 344 - protein, 7 aa, Homo sapiens
HKNNRPS

SEQ ID NO: 345 - protein, 7 aa, Homo sapiens
GHNNRPS

SEQ ID NO: 346 - protein, 7 aa, Homo sapiens
GKHNRPS

SEQ ID NO: 347 - protein, 7 aa, Homo sapiens
GKNHRPS

SEQ ID NO: 348 - protein, 7 aa, Homo sapiens
GKNNHPS

SEQ ID NO: 349 - protein, 7 aa, Homo sapiens
GKNNRHS

SEQ ID NO: 350 - protein, 7 aa, Homo sapiens
GKNNRPH

SEQ ID NO: 351 - protein, 7 aa, Homo sapiens
KKNNRPS

SEQ ID NO: 352 - protein, 7 aa, Homo sapiens
GKKNRPS

SEQ ID NO: 353 - protein, 7 aa, Homo sapiens
GKNKRPS

SEQ ID NO: 354 - protein, 7 aa, Homo sapiens
GKNNKPS

SEQ ID NO: 355 - protein, 7 aa, Homo sapiens
GKNNRKS

SEQ ID NO: 356 - protein, 7 aa, Homo sapiens
GKNNRPK

SEQ ID NO: 357 - protein, 7 aa, Homo sapiens
LKNNRPS

SEQ ID NO: 358 - protein, 7 aa, Homo sapiens
GLNNRPS

SEQ ID NO: 359 - protein, 7 aa, Homo sapiens
GKLNRPS

SEQ ID NO: 360 - protein, 7 aa, Homo sapiens
GKNLRPS

SEQ ID NO: 361 - protein, 7 aa, Homo sapiens
GKNNLPS

SEQ ID NO: 362 - protein, 7 aa, Homo sapiens
GKNNRLS

SEQ ID NO: 363 - protein, 7 aa, Homo sapiens
GKNNRPL

SEQ ID NO: 364 - protein, 7 aa, Homo sapiens
QKNNRPS

SEQ ID NO: 365 - protein, 7 aa, Homo sapiens
GQNNRPS

SEQ ID NO: 366 - protein, 7 aa, Homo sapiens
GKQNRPS

SEQ ID NO: 367 - protein, 7 aa, Homo sapiens
GKNQRPS

SEQ ID NO: 368 - protein, 7 aa, Homo sapiens
GKNNQPS

SEQ ID NO: 369 - protein, 7 aa, Homo sapiens
GKNNRQS

SEQ ID NO: 370 - protein, 7 aa, Homo sapiens
GKNNRPQ

SEQ ID NO: 371 - protein, 7 aa, Homo sapiens
SKNNRPS

SEQ ID NO: 372 - protein, 7 aa, Homo sapiens
GSNNRPS

SEQ ID NO: 373 - protein, 7 aa, Homo sapiens
GKSNRPS

SEQ ID NO: 374 - protein, 7 aa, Homo sapiens
GKNSRPS

SEQ ID NO: 375 - protein, 7 aa, Homo sapiens
GKNNSPS

SEQ ID NO: 376 - protein, 7 aa, Homo sapiens
GKNNRSS

SEQ ID NO: 377 - protein, 7 aa, Homo sapiens
WKNNRPS

SEQ ID NO: 378 - protein, 7 aa, Homo sapiens
GWNNRPS

SEQ ID NO: 379 - protein, 7 aa, Homo sapiens
GKWNRPS

SEQ ID NO: 380 - protein, 7 aa, Homo sapiens
GKNWRPS

SEQ ID NO: 381 - protein, 7 aa, Homo sapiens
GKNNWPS

SEQ ID NO: 382 - protein, 7 aa, Homo sapiens
GKNNRWS

SEQ ID NO: 383 - protein, 7 aa, Homo sapiens
GKNNRPW

SEQ ID NO: 384 - protein, 7 aa, Homo sapiens
YKNNRPS

SEQ ID NO: 385 - protein, 7 aa, Homo sapiens
GYNNRPS

SEQ ID NO: 386 - protein, 7 aa, Homo sapiens
GKYNRPS

SEQ ID NO: 387 - protein, 7 aa, Homo sapiens
GKNYRPS

SEQ ID NO: 388 - protein, 7 aa, Homo sapiens
GKNNYPS

SEQ ID NO: 389 - protein, 7 aa, Homo sapiens
GKNNRYS

SEQ ID NO: 390 - protein, 7 aa, Homo sapiens
GKNNRPY

SEQ ID NO: 391 - protein, 11 aa, Homo sapiens
NARDSSGKNLV

SEQ ID NO: 392 - protein, 11 aa, Homo sapiens
NSRDASGKNLV

SEQ ID NO: 393 - protein, 11 aa, Homo sapiens
NSRDSAGKNLV

SEQ ID NO: 394 - protein, 11 aa, Homo sapiens
NSRDSSAKNLV

SEQ ID NO: 395 - protein, 11 aa, Homo sapiens
NSRDSSGANLV

SEQ ID NO: 396 - protein, 11 aa, Homo sapiens
NSRDSSGKALV

SEQ ID NO: 397 - protein, 11 aa, Homo sapiens
NSRDSSGKNAV

SEQ ID NO: 398 - protein, 11 aa, Homo sapiens
NSRDSSGKNLA

SEQ ID NO: 399 - protein, 11 aa, Homo sapiens
DSRDSSGKNLV

SEQ ID NO: 400 - protein, 11 aa, Homo sapiens
NDRDSSGKNLV

SEQ ID NO: 401 - protein, 11 aa, Homo sapiens
NSRDDSGKNLV

SEQ ID NO: 402 - protein, 11 aa, Homo sapiens
NSRDSDGKNLV

SEQ ID NO: 403 - protein, 11 aa, Homo sapiens
NSRDSSGDNLV

SEQ ID NO: 404 - protein, 11 aa, Homo sapiens
NSRDSSGKDLV

SEQ ID NO: 405 - protein, 11 aa, Homo sapiens
NSRDSSGKNLD

SEQ ID NO: 406 - protein, 11 aa, Homo sapiens
HSRDSSGKNLV

SEQ ID NO: 407 - protein, 11 aa, Homo sapiens
NSRDHSGKNLV

SEQ ID NO: 408 - protein, 11 aa, Homo sapiens
NSRDSHGKNLV

SEQ ID NO: 409 - protein, 11 aa, Homo sapiens
NSRDSSGHNLV

SEQ ID NO: 410 - protein, 11 aa, Homo sapiens
NSRDSSGKHLV

SEQ ID NO: 411 - protein, 11 aa, Homo sapiens
NSRDSSGKNHV

SEQ ID NO: 412 - protein, 11 aa, Homo sapiens
NSRDSSGKNLH

SEQ ID NO: 413 - protein, 11 aa, Homo sapiens
KSRDSSGKNLV

SEQ ID NO: 414 - protein, 11 aa, Homo sapiens
NSKDSSGKNLV

SEQ ID NO: 415 - protein, 11 aa, Homo sapiens
NSRDKSGKNLV

SEQ ID NO: 416 - protein, 11 aa, Homo sapiens
NSRDSKGKNLV

SEQ ID NO: 417 - protein, 11 aa, Homo sapiens
NSRDSSGKKLV

SEQ ID NO: 418 - protein, 11 aa, Homo sapiens
NSRDSSGKNLK

SEQ ID NO: 419 - protein, 11 aa, Homo sapiens
LSRDSSGKNLV

SEQ ID NO: 420 - protein, 11 aa, Homo sapiens
NSRDLSGKNLV

SEQ ID NO: 421 - protein, 11 aa, Homo sapiens
NSRDSLGKNLV

SEQ ID NO: 422 - protein, 11 aa, Homo sapiens
NSRDSSLKNLV

SEQ ID NO: 423 - protein, 11 aa, Homo sapiens
NSRDSSGLNLV

SEQ ID NO: 424 - protein, 11 aa, Homo sapiens
NSRDSSGKLLV

SEQ ID NO: 425 - protein, 11 aa, Homo sapiens
NSRDSSGKNLL

SEQ ID NO: 426 - protein, 11 aa, Homo sapiens
QSRDSSGKNLV

SEQ ID NO: 427 - protein, 11 aa, Homo sapiens
NSRDQSGKNLV

SEQ ID NO: 428 - protein, 11 aa, Homo sapiens
NSRDSQGKNLV

SEQ ID NO: 429 - protein, 11 aa, Homo sapiens
NSRDSSGQNLV

SEQ ID NO: 430 - protein, 11 aa, Homo sapiens
NSRDSSGKQLV

SEQ ID NO: 431 - protein, 11 aa, Homo sapiens
NSRDSSGKNQV

SEQ ID NO: 432 - protein, 11 aa, Homo sapiens
NSRDSSGKNLQ

SEQ ID NO: 433 - protein, 11 aa, Homo sapiens
SSRDSSGKNLV

SEQ ID NO: 434 - protein, 11 aa, Homo sapiens
NSRDSSSKNLV

SEQ ID NO: 435 - protein, 11 aa, Homo sapiens
NSRDSSGSNLV

SEQ ID NO: 436 - protein, 11 aa, Homo sapiens
NSRDSSGKSLV

SEQ ID NO: 437 - protein, 11 aa, Homo sapiens
NSRDSSGKNSV

SEQ ID NO: 438 - protein, 11 aa, Homo sapiens
NSRDSSGKNLS

SEQ ID NO: 439 - protein, 11 aa, Homo sapiens
NSRDWSGKNLV

SEQ ID NO: 440 - protein, 11 aa, Homo sapiens
NSRDSWGKNLV

SEQ ID NO: 441 - protein, 11 aa, Homo sapiens
NSRDSSGWNLV

SEQ ID NO: 442 - protein, 11 aa, Homo sapiens
NSRDSSGKWLV

SEQ ID NO: 443 - protein, 11 aa, Homo sapiens
NSRDSSGKNWV

SEQ ID NO: 444 - protein, 11 aa, Homo sapiens
NSRDSSGKNLW

SEQ ID NO: 445 - protein, 11 aa, Homo sapiens
YSRDSSGKNLV

SEQ ID NO: 446 - protein, 11 aa, Homo sapiens
NSRDYSGKNLV

SEQ ID NO: 447 - protein, 11 aa, Homo sapiens
NSRDSYGKNLV

SEQ ID NO: 448 - protein, 11 aa, Homo sapiens
NSRDSSYKNLV

SEQ ID NO: 449 - protein, 11 aa, Homo sapiens
NSRDSSGYNLV

SEQ ID NO: 450 - protein, 11 aa, Homo sapiens
NSRDSSGKYLV

SEQ ID NO: 451 - protein, 11 aa, Homo sapiens
NSRDSSGKNYV

SEQ ID NO: 452 - protein, 11 aa, Homo sapiens
NSRDSSGKNLY

SEQ ID NO: 453 - protein, 11 aa, Homo sapiens
GGSISSSNWWS

SEQ ID NO: 454 - protein, 119 aa, Homo sapiens
QVQLQESGPGLVKPSGTLSLTCAVSGGSISSSNWWSWVRQPPGKGLEWIGEIYHYGYTNYNPSLKSRVTISVDKSKNQFSLKLISVTAADTAVYYCAREGIGWPSFDYWGQGTLVTVSS

SEQ ID NO: 455 - protein, 108 aa, Homo sapiens
SSELTQDPAASVALGQTVRITCQGDTLRSYYASWYQQKPGQAPILVIYGKNNRPSGIPDRFSGSSSGNTASLTITGAQAEDEADYYCNSRDSSGKNLVFGGGTKLTVL

SEQ ID NO: 456 - protein, 214 aa, Homo sapiens
SSELTQDPAASVALGQTVRITCQGDTLRSYYASWYQQKPGQAPILVIYGKNNRPSGIPDRFSGSSSGNTASLTITGAQAEDEADYYCNSRDSSGKNLVFGGGTKLTVLGQPKAAPSVTLFPPSSEELQANKATLVCLISDFYPGAVTVAWKADSSPVKAGVETTTPSKQSNNKYAASSYLSLTPEQWKSHRSYSCQVTHEGSTVEKTVAPTECS

SEQ ID NO: 457 - protein, 108 aa, Homo sapiens
SSELTQDPAASVALGQTVRITCQGDTLRNYYASWYQQKPGQAPILVIYGKNNRPSGIPDRFSGSSSGNTASLTITGAQAEDEADYYCNSRDLSGKNLVFGGGTKLTVL

SEQ ID NO: 458 - protein, 214 aa, Homo sapiens
SSELTQDPAASVALGQTVRITCQGDTLRNYYASWYQQKPGQAPILVIYGKNNRPSGIPDRFSGSSSGNTASLTITGAQAEDEADYYCNSRDLSGKNLVFGGGTKLTVLGQPKAAPSVTLFPPSSEELQANKATLVCLISDFYPGAVTVAWKADSSPVKAGVETTTPSKQSNNKYAASSYLSLTPEQWKSHRSYSCQVTHEGSTVEKTVAPTECS

SEQ ID NO: 459 - protein, 108 aa, Homo sapiens
SSELTQDPAASVALGQTVRITCQGDTLRNYYASWYQQKPGQAPILVIYGKNNRPSGIPDRFSGSSSGNTASLTITGAQAEDEADYYCNSRDFSGKNLVFGGGTKLTVL

SEQ ID NO: 460 - protein, 214 aa, Homo sapiens
SSELTQDPAASVALGQTVRITCQGDTLRNYYASWYQQKPGQAPILVIYGKNNRPSGIPDRFSGSSSGNTASLTITGAQAEDEADYYCNSRDFSGKNLVFGGGTKLTVLGQPKAAPSVTLFPPSSEELQANKATLVCLISDFYPGAVTVAWKADSSPVKAGVETTTPSKQSNNKYAASSYLSLTPEQWKSHRSYSCQVTHEGSTVEKTVAPTECS

SEQ ID NO: 461 - protein, 119 aa, Homo sapiens; identical to SEQ ID NO: 7

SEQ ID NO: 462 - protein, 119 aa, Homo sapiens
QVQLQESGPGLVKPSGTLSLTCAVSGGSISSSNWWSWVRQPPGKGLEWIGEIYHFGNTNYNPSLKSRVTISVDKSKNQFSLKLISVTAADTAVYYCAREGIGWPSFDYWGQGTLVTVSS

SEQ ID NO: 463 - protein, 119 aa, Homo sapiens
QVQLQESGPGLVKPSGTLSLTCAVSGGSISSSNWWSWVRQPPGKGLEWIGEIYHYGNTNYNPSLKSRVTISVDKSKNQFSLKLISVTAADTAVYYCAREGIGWPSFDYWGQGTLVTVSS

SEQ ID NO: 464 - protein, 119 aa, Homo sapiens
QVQLQESGPGLVKPSGTLSLTCAVSGGSISSSNWWSWVRQPPGKGLEWIGEIYHWGNTNYNPSLKSRVTISVDKSKNQFSLKLISVTAADTAVYYCAREGIGWPSFDYWGQGTLVTVSS

SEQ ID NO: 465 - protein, 119 aa, Homo sapiens
QVQLQESGPGLVKPSGTLSLTCAVSGGSISSSNWWSWVRQPPGKGLEWIGEIYHSGWTNYNPSLKSRVTISVDKSKNQFSLKLISVTAADTAVYYCAREGIGWPSFDYWGQGTLVTVSS

SEQ ID NO: 466 - protein, 119 aa, Homo sapiens
QVQLQESGPGLVKPSGTLSLTCAVSGGSISSSNWWSWVRQPPGKGLEWIGEIYHFGFTNYNPSLKSRVTISVDKSKNQFSLKLISVTAADTAVYYCAREGIGWPSFDYWGQGTLVTVSS

SEQ ID NO: 467 - protein, 119 aa, Homo sapiens
QVQLQESGPGLVKPSGTLSLTCAVSGGSISSSNWWSWVRQPPGKGLEWIGEIYHYGFTNYNPSLKSRVTISVDKSKNQFSLKLISVTAADTAVYYCAREGIGWPSFDYWGQGTLVTVSS

SEQ ID NO: 468 - protein, 119 aa, Homo sapiens
QVQLQESGPGLVKPSGTLSLTCAVSGGSISSSNWWSWVRQPPGKGLEWIGEIYHWGFTNYNPSLKSRVTISVDKSKNQFSLKLISVTAADTAVYYCAREGIGWPSFDYWGQGTLVTVSS

SEQ ID NO: 469 - protein, 119 aa, Homo sapiens
QVQLQESGPGLVKPSGTLSLTCAVSGGSISSSNWWSWVRQPPGKGLEWIGEIYHFGYTNYNPSLKSRVTISVDKSKNQFSLKLISVTAADTAVYYCAREGIGWPSFDYWGQGTLVTVSS

SEQ ID NO: 470 - protein, 119 aa, Homo sapiens; identical to SEQ ID NO: 454

SEQ ID NO: 471 - protein, 119 aa, Homo sapiens
QVQLQESGPGLVKPSGTLSLTCAVSGGSISSSNWWSWVRQPPGKGLEWIGEIYHWGYTNYNPSLKSRVTISVDKSKNQFSLKLISVTAADTAVYYCAREGIGWPSFDYWGQGTLVTVSS

SEQ ID NO: 472 - protein, 119 aa, Homo sapiens
QVQLQESGPGLVKPSGTLSLTCAVSGGSISSSNWWSWVRQPPGKGLEWIGEIYHFGWTNYNPSLKSRVTISVDKSKNQFSLKLISVTAADTAVYYCAREGIGWPSFDYWGQGTLVTVSS

SEQ ID NO: 473 - protein, 119 aa, Homo sapiens
QVQLQESGPGLVKPSGTLSLTCAVSGGSISSSNWWSWVRQPPGKGLEWIGEIYHYGWTNYNPSLKSRVTISVDKSKNQFSLKLISVTAADTAVYYCAREGIGWPSFDYWGQGTLVTVSS

SEQ ID NO: 474 - protein, 119 aa, Homo sapiens
QVQLQESGPGLVKPSGTLSLTCAVSGGSISSSNWWSWVRQPPGKGLEWIGEIYHWGWTNYNPSLKSRVTISVDKSKNQFSLKLISVTAADTAVYYCAREGIGWPSFDYWGQGTLVTVSS

SEQ ID NO: 475 - protein, 119 aa, Homo sapiens
QVQLQESGPGLVKPSGTLSLTCAVSGGSISSSNWWAWVRQPPGKGLEWIGEIYHSGNTNYNPSLKSRVTISVDKSKNQFSLKLISVTAADTAVYYCAREGIGWPSFDYWGQGTLVTVSS

SEQ ID NO: 476 - protein, 119 aa, Homo sapiens
QVQLQESGPGLVKPSGTLSLTCAVSGGSISSSNWLSWVRQPPGKGLEWIGEIYHSGNTNYNPSLKSRVTISVDKSKNQFSLKLISVTAADTAVYYCAREGIGWPSFDYWGQGTLVTVSS

SEQ ID NO: 477 - protein, 119 aa, Homo sapiens
QVQLQESGPGLVKPSGTLSLTCAVSGGSISSSNWWSWVRQPPGKGLEWIGEIWHSGNTNYNPSLKSRVTISVDKSKNQFSLKLISVTAADTAVYYCAREGIGWPSFDYWGQGTLVTVSS

SEQ ID NO: 478 - protein, 119 aa, Homo sapiens
QVQLQESGPGLVKPSGTLSLTCAVSGGSISSSNWWSWVRQPPGKGLEWIGEIYHSGHTNYNPSLKSRVTISVDKSKNQFSLKLISVTAADTAVYYCAREGIGWPSFDYWGQGTLVTVSS

SEQ ID NO: 479 - protein, 119 aa, Homo sapiens
QVQLQESGPGLVKPSGTLSLTCAVSGGSISSSNWWSWVRQPPGKGLEWIGEIYHSGLTNYNPSLKSRVTISVDKSKNQFSLKLISVTAADTAVYYCAREGIGWPSFDYWGQGTLVTVSS

SEQ ID NO: 480 - protein, 119 aa, Homo sapiens
QVQLQESGPGLVKPSGTLSLTCAVSGGSISSSNWWSWVRQPPGKGLEWIGEIYHSGNDNYNPSLKSRVTISVDKSKNQFSLKLISVTAADTAVYYCAREGIGWPSFDYWGQGTLVTVSS

SEQ ID NO: 481 - protein, 119 aa, Homo sapiens
QVQLQESGPGLVKPSGTLSLTCAVSGGSISSSNWWSWVRQPPGKGLEWIGEIYHSGNTQYNPSLKSRVTISVDKSKNQFSLKLISVTAADTAVYYCAREGIGWPSFDYWGQGTLVTVSS

SEQ ID NO: 482 - protein, 119 aa, Homo sapiens
QVQLQESGPGLVKPSGTLSLTCAVSGGSISSSNWWSWVRQPPGKGLEWIGEIYHSGNTNYYPSLKSRVTISVDKSKNQFSLKLISVTAADTAVYYCAREGIGWPSFDYWGQGTLVTVSS

SEQ ID NO: 483 - protein, 119 aa, Homo sapiens
QVQLQESGPGLVKPSGTLSLTCAVSGGSISSSNWWSWVRQPPGKGLEWIGEIYHSGNTNYNPSLKSRVTISVDKSKNQFSLKLISVTAADTAVYYCAREGIGWPSFDSWGQGTLVTVSS

SEQ ID NO: 484 - protein, 119 aa, Homo sapiens
QVQLQESGPGLVKPSGTLSLTCAVSGGSISSSNWWSWVRQPPGKGLEWIGEIYHSGNTNYNPSLKSRVTISVDKSKNQFSLKLISVTAADTAVYYCAREGIGWPSFDLWGQGTLVTVSS

SEQ ID NO: 485 - protein, 119 aa, Homo sapiens
QVQLQESGPGLVKPSGTLSLTCAVSGGSISSSNWWSWVRQPPGKGLEWIGEIYHSGNTNYNPSLKSRVTISVDKSKNQFSLKLISVTAADTAVYYCAREGIGWPSFDAWGQGTLVTVSS

SEQ ID NO: 486 - protein, 119 aa, Homo sapiens
QVQLQESGPGLVKPSGTLSLTCAVSGGSISSSNWWSWVRQPPGKGLEWIGEIYHSGNTNYNPSLKSRVTISVDKSKNQFSLKLISVTAADTAVYYCAREGIGWPSFDHWGQGTLVTVSS

SEQ ID NO: 487 - protein, 119 aa, Homo sapiens
QVQLQESGPGLVKPSGTLSLTCAVSGGSISSSNWWSWVRQPPGKGLEWIGEIYHWGWTNYYPSLKSRVTISVDKSKNQFSLKLISVTAADTAVYYCAREGIGWPSFDYWGQGTLVTVSS

SEQ ID NO: 488 - protein, 119 aa, Homo sapiens
QVQLQESGPGLVKPSGTLSLTCAVSGGSISSSNWWSWVRQPPGKGLEWIGEIYHSGNTNYNPSLKSRVTISVDKSKNQFSLKLSSVTAADTAVYYCAREGIGWPSFDYWGQGTLVTVSS

SEQ ID NO: 489 - protein, 119 aa, Homo sapiens
QVQLQESGPGLVKPSGTLSLTCAVSGGSISSSNWWSWVRQPPGKGLEWIGEIYHYGWTNYNPSLKSRVTISVDKSKNQFSLKLSSVTAADTAVYYCAREGIGWPSFDYWGQGTLVTVSS

SEQ ID NO: 490 - protein, 119 aa, Homo sapiens; identical to SEQ ID NO: 4

SEQ ID NO: 491 - protein, 108 aa, Homo sapiens; identical to SEQ ID NO: 8

SEQ ID NO: 492 - protein, 108 aa, Homo sapiens
SSELTQDPAASVALGQTVRITCQGDTLRNYYASWYQQKPGQAPILVIYGKNNRPSGIPDRFSGSSSGNTASLTITGAQAEDEADYYCNSRSSSGKNLVFGGGTKLTVL

SEQ ID NO: 493 - protein, 108 aa, Homo sapiens
SSELTQDPAASVALGQTVRITCQGDTLRNYYASWYQQKPGQAPILVIYSKNNRPSGIPDRFSGSSSGNTASLTITGAQAEDEADYYCNSRDSSGKNLVFGGGTKLTVL

SEQ ID NO: 494 - protein, 108 aa, Homo sapiens
SSELTQDPAASVALGQTVRITCQGDTLRNYYASWYQQKPGQAPILVIYGANNRPSGIPDRFSGSSSGNTASLTITGAQAEDEADYYCNSRDSSGKNLVFGGGTKLTVL

SEQ ID NO: 495 - protein, 108 aa, Homo sapiens
SSELTQDPAASVALGQTVRITCQGDTLRNYYASWYQQKPGQAPILVIYGHNNRPSGIPDRFSGSSSGNTASLTITGAQAEDEADYYCNSRDSSGKNLVFGGGTKLTVL

SEQ ID NO: 496 - protein, 108 aa, Homo sapiens
SSELTQDPAASVALGQTVRITCQGDTLRNYYASWYQQKPGQAPILVIYGLNNRPSGIPDRFSGSSSGNTASLTITGAQAEDEADYYCNSRDSSGKNLVFGGGTKLTVL

SEQ ID NO: 497 - protein, 108 aa, Homo sapiens
SSELTQDPAASVALGQTVRITCQGDTLRNYYASWYQQKPGQAPILVIYGKNNLPSGIPDRFSGSSSGNTASLTITGAQAEDEADYYCNSRDSSGKNLVFGGGTKLTVL

SEQ ID NO: 498 - protein, 108 aa, Homo sapiens
SSELTQDPAASVALGQTVRITCQGDTLRNYYASWYQQKPGQAPILVIYGKNNQPSGIPDRFSGSSSGNTASLTITGAQAEDEADYYCNSRDSSGKNLVFGGGTKLTVL

SEQ ID NO: 499 - protein, 108 aa, Homo sapiens
SSELTQDPAASVALGQTVRITCQGDTLRNYYASWYQQKPGQAPILVIYGKNNYPSGIPDRFSGSSSGNTASLTITGAQAEDEADYYCNSRDSSGKNLVFGGGTKLTVL

SEQ ID NO: 500 - protein, 108 aa, Homo sapiens
SSELTQDPAASVALGQTVRITCQGDTLRNYYASWYQQKPGQAPILVIYGHNNLPSGIPDRFSGSSSGNTASLTITGAQAEDEADYYCNSRDSSGKNLVFGGGTKLTVL

SEQ ID NO: 501 - protein, 108 aa, Homo sapiens
SSELTQDPAASVALGQTVRITCQGDTLRNYYASWYQQKPGQAPILVIYGHNNYPSGIPDRFSGSSSGNTASLTITGAQAEDEADYYCNSRDSSGKNLVFGGGTKLTVL

SEQ ID NO: 502 - protein, 108 aa, Homo sapiens; identical to SEQ ID NO: 455

SEQ ID NO: 503 - protein, 108 aa, Homo sapiens
SSELTQDPAASVALGQTVRITCQGDTLRNYYASWYQQKPGQAPILVIYGKNNRPSGIPDRFSGSSSGNTASLTITGAQAEDEADYYCNSRESSGKNLVFGGGTKLTVL

SEQ ID NO: 504 - protein, 108 aa, Homo sapiens; identical to SEQ ID NO: 457

SEQ ID NO: 505 - protein, 108 aa, Homo sapiens
SSELTQDPAASVALGQTVRITCQGDTLRNYYASWYQQKPGQAPILVIYGKNNRPSGIPDRFSGSSSGNTASLTITGAQAEDEADYYCNSRDESGKNLVFGGGTKLTVL

SEQ ID NO: 506 - protein, 108 aa, Homo sapiens; identical to SEQ ID NO: 459

SEQ ID NO: 507 - protein, 108 aa, Homo sapiens
SSELTQDPAASVALGQTVRITCQGDTLRSYYASWYQQKPGQAPILVIYGKNNRPSGIPDRFSGSSSGNTASLTITGAQAEDEADYYCNSRESSGKNLVFGGGTKLTVL

SEQ ID NO: 508 - protein, 108 aa, Homo sapiens; identical to SEQ ID NO: 5

SEQ ID NO: 509 - protein, 108 aa, Homo sapiens
SSELTQDPAASVALGQTVRITCQGDTLRSYYASWYQQKPGQAPILVIYGKNNRPSGIPDRFSGSSSGNTASLTITGAQAEDEADYYCNSRDESGKNLVFGGGTKLTVL

SEQ ID NO: 510 - protein, 108 aa, Homo sapiens
SSELTQDPAASVALGQTVRITCQGDTLRSYYASWYQQKPGQAPILVIYGKNNRPSGIPDRFSGSSSGNTASLTITGAQAEDEADYYCNSRDFSGKNLVFGGGTKLTVL

SEQ ID NO: 511 - protein, 114 aa, Homo sapiens
NWVNVISDLKKIEDLIQSMHIDATLYTESDVHPSCKVTAMKCFLLELQVISLESGDASIHDTVENLIILANNSLSSNGNVTESGCKECEELEEKNIKEFLQSFVHIVQMFINTS

SEQ ID NO: 512 - protein, 211 aa, Homo sapiens
ITCPPPMSVEHADIWVKSYSLYSRERYICNSGFKRKAGTSSLTECVLNKATNVAHWTTPSLKCIRDPALVHQRPAPPSTVTTAGVTPQPESLSPSGKEPAASSPSSNNTAATTAAIVPGSQLMPSKSPSTGTTEISSHESSHGTPSQTTAKNWELTASASHQPPGVYPQGHSDTTKRVGSIEGRGSGLNDIFEAQKIEWHEGSHHHHHHHH

SEQ ID NO: 513 - protein, 107 aa, Homo sapiens [sequence omitted]

SEQ ID NO: 514 - protein, 106 aa, Homo sapiens
GQPKAAPSVTLFPPSSEELQANKATLVCLISDFYPGAVTVAWKADSSPVKAGVETTTPSKQSNNKYAASSYLSLTPEQWKSHRSYSCQVTHEGSTVEKTVAPTECS

SEQ ID NO: 515 - protein, 448 aa, Homo sapiens
EVQLVQSGAEVKKPGESLKISCKVSGYFFTTYWIGWVRQMPGKGLEYMGIIYPGDSDTRYSPSFQGQVTISADKSISTAYLQWSSLKASDTAMYYCARGGNWNCFDYWGQGTLVTVSSASTKGPSVFPLAPSSKSTSGGTAALGCLVKDYFPEPVTVSWNSGALTSGVHTFPAVLQSSGLYSLSSVVTVPSSSLGTQTYICNVNHKPSNTKVDKKVEPKSCDKTHTCPPCPAPELLGGPSVFLFPPKPKDTLMISRTPEVTCVVVDVSHEDPEVKFNWYVDGVEVHNAKTKPREEQYNSTYRVVSVLTVLHQDWLNGKEYKCKVSNKALPAPIEKTISKAKGQPREPQVYTLPPSRDELTKNQVSLTCLVKGFYPSDIAVEWESNGQPENNYKTTPPVLDSDGSFFLYSKLTVDKSRWQQGNVFSCSVMHEALHNHYTQKSLSLSPGK

SEQ ID NO: 516 - protein, 214 aa, Homo sapiens
EIVLTQSPGTLSLSPGERATLSCRASQSVSSSYLAWYQQKPGQAPRLLIYGASRRATGIPDRFSGSGSGTDFTLTISRLEPEDFAVYYCQRYGSSHTFGQGTKLEISRTVAAPSVFIFPPSDEQLKSGTASVVCLLNNFYPREAKVQWKVDNALQSGNSQESVTEQDSKDSTYSLSSTLTLSKADYEKHKVYACEVTHQGLSSPVTKSFNRGEC

SEQ ID NO: 517 - DNA, 357 bp, Homo sapiens
caggtgcagctgcaggaatctggccccggactggtgaaacctagcggcaccctgagcctgacctgcgccgtgagcggcggcagcatcagcagcagcaactggtggagctgggtccgccagcctcctggcaagggcctggaatggatcggcgagatctaccactacggctacaccaactacaaccccagcctgaagtcccgggtgaccatcagcgtggacaagagcaagaaccagttcagcctgaagctgtccagcgtgacagccgccgacaccgccgtgtactactgcgccagagagggaatcggctggcccagcttcgattactggggccagggcaccctggtgacagtgtcctca

SEQ ID NO: 518 - DNA, 327 bp, Homo sapiens
agcagcgagctgacccaggatcccgctgcttccgtggctctgggccagaccgtgcggatcacctgtcagggcgacaccctgcggagctactacgccagctggtatcagcagaagcccggccaggcccccatcctggtgatctacggcaagaacaaccggcccagcggcatccccgacagattcagcggcagcagcagcggcaacaccgccagcctgaccatcactggcgctcaggccgaggacgaggccgactactactgcaacagccgggacctttccggcaagaacctggtgttcggcggaggcaccaagctgaccgtcctaggt

SEQ ID NO: 519 - protein, 11 aa, Homo sapiens
NSRDFSGKNLV

SEQ ID NO: 520 - protein, 186 aa, Homo sapiens
ITCPPPMSVEHADIWVKSYSLYSRERYICNSGFKRKAGTSSLTECVLNKATNVAHWTTPSLKCIRDPALVHQRPAPPSTVTTAGVTPQPESLSPSGKEPAASSPSSNNTAATTAAIVPGSQLMPSKSPSTGTTEISSHESSHGTPSQTTAKNWELTASASHQPPGVYPQGHSDTTKRVGSIEGRGS